European Patent Application EP 4 372 085 A1, published May 22, 2024. Title: NUCLEIC ACID, COMPOSITION AND CONJUGATE CONTAINING SAME, AND PREPARATION METHOD AND USE. Applicant: SUZHOU RIBO LIFE SCIENCE CO., LTD. The sequence listing filed with the application follows.

SEQUENCE LISTING (170 sequences)

SEQ ID NO: 1 - RNA, 19 nt, Artificial Sequence
  siRNA
  misc_feature (19)..(19): n is Z1, and Z1 is A
caauaaagcuggacaagan

SEQ ID NO: 2 - RNA, 19 nt, Artificial Sequence
  siRNA
  misc_feature (1)..(1): n is Z2, and Z2 is U
nucuuguccagcuuuauug

SEQ ID NO: 3 - RNA, 19 nt, Artificial Sequence
  siRNA
  misc_feature (19)..(19): n is Z3, and Z3 is selected from A, U, G or C
caauaaagcuggacaagan

SEQ ID NO: 4 - RNA, 19 nt, Artificial Sequence
  siRNA
  misc_feature (1)..(1): n is Z4, Z4 is a nucleotide complementary to Z3, and Z3 is selected from A, U, G or C
nucuuguccagcuuuauug

SEQ ID NO: 5 - RNA, 19 nt, Artificial Sequence
  siRNA
  misc_feature (19)..(19): n is Z3, and Z3 is selected from A, U, G or C
caauaaagcuggacaagan

SEQ ID NO: 6 - RNA, 21 nt, Artificial Sequence
  siRNA
  misc_feature (1)..(1): n is Z4, Z4 is a nucleotide complementary to Z3, and Z3 is selected from A, U, G or C
nucuuguccagcuuuauuggg

SEQ ID NO: 7 - RNA, 21 nt, Artificial Sequence
  siRNA
  misc_feature (21)..(21): n is Z3, and Z3 is selected from A, U, G or C
cccaauaaagcuggacaagan

SEQ ID NO: 8 - RNA, 23 nt, Artificial Sequence
  siRNA
  misc_feature (1)..(1): n is Z4, Z4 is a nucleotide complementary to Z3, and Z3 is selected from A, U, G or C
nucuuguccagcuuuauugggag

SEQ ID NO: 9 - RNA, 19 nt, Artificial Sequence
  siRNA
caauaaagcuggacaagaa

SEQ ID NO: 10 - RNA, 21 nt, Artificial Sequence
  siRNA
uucuuguccagcuuuauuggg

SEQ ID NO: 11 - RNA, 21 nt, Artificial Sequence
  siRNA
cccaauaaagcuggacaagaa

SEQ ID NO: 12 - RNA, 23 nt, Artificial Sequence
  siRNA
uucuuguccagcuuuauugggag

SEQ ID NO: 13 - RNA, 19 nt, Artificial Sequence
  siRNA
caauaaagcuggacaagaa

SEQ ID NO: 14 - RNA, 21 nt, Artificial Sequence
  siRNA
uucuuguccagcuuuauuggg

SEQ ID NO: 15 - RNA, 19 nt, Artificial Sequence
  siRNA
caauaaagcuggacaagaa

SEQ ID NO: 16 - RNA, 21 nt, Artificial Sequence
  siRNA
uucuuguccagcuuuauuggg

SEQ ID NO: 17 - RNA, 21 nt, Artificial Sequence
  siRNA
cccaauaaagcuggacaagaa

SEQ ID NO: 18 - RNA, 23 nt, Artificial Sequence
  siRNA
uucuuguccagcuuuauugggag

SEQ ID NO: 19 - RNA, 21 nt, Artificial Sequence
  siRNA
cccaauaaagcuggacaagaa

SEQ ID NO: 20 - RNA, 23 nt, Artificial Sequence
  siRNA
uucuuguccagcuuuauugggag

SEQ ID NO: 21 - RNA, 19 nt, Artificial Sequence
  siRNA
caauaaagcuggacaagaa

SEQ ID NO: 22 - RNA, 21 nt, Artificial Sequence
  siRNA
uucuuguccagcuuuauuggg

SEQ ID NO: 23 - RNA, 19 nt, Artificial Sequence
  siRNA
caauaaagcuggacaagaa

SEQ ID NO: 24 - RNA, 21 nt, Artificial Sequence
  siRNA
uucuuguccagcuuuauuggg

SEQ ID NO: 25 - RNA, 21 nt, Artificial Sequence
  siRNA
cccaauaaagcuggacaagaa

SEQ ID NO: 26 - RNA, 23 nt, Artificial Sequence
  siRNA
uucuuguccagcuuuauugggag

SEQ ID NO: 27 - RNA, 21 nt, Artificial Sequence
  siRNA
cccaauaaagcuggacaagaa

SEQ ID NO: 28 - RNA, 23 nt, Artificial Sequence
  siRNA
uucuuguccagcuuuauugggag

SEQ ID NO: 29 - RNA, 19 nt, Artificial Sequence
  siRNA
caauaaagcuggacaagaa

SEQ ID NO: 30 - RNA, 21 nt, Artificial Sequence
  siRNA
uucuuguccagcuuuauuggg

SEQ ID NO: 31 - RNA, 19 nt, Artificial Sequence
  siRNA
caauaaagcuggacaagaa

SEQ ID NO: 32 - RNA, 21 nt, Artificial Sequence
  siRNA
uucuuguccagcuuuauuggg

SEQ ID NO: 33 - RNA, 21 nt, Artificial Sequence
  siRNA
cccaauaaagcuggacaagaa

SEQ ID NO: 34 - RNA, 23 nt, Artificial Sequence
  siRNA
uucuuguccagcuuuauugggag

SEQ ID NO: 35 - RNA, 21 nt, Artificial Sequence
  siRNA
cccaauaaagcuggacaagaa

SEQ ID NO: 36 - RNA, 23 nt, Artificial Sequence
  siRNA
uucuuguccagcuuuauugggag

SEQ ID NO: 37 - RNA, 19 nt, Artificial Sequence
  siRNA
caauaaagcuggacaagaa

SEQ ID NO: 38 - RNA, 21 nt, Artificial Sequence
  siRNA
uucuuguccagcuuuauuggg

SEQ ID NO: 39 - RNA, 19 nt, Artificial Sequence
  siRNA
caauaaagcuggacaagaa

SEQ ID NO: 40 - RNA, 21 nt, Artificial Sequence
  siRNA
uucuuguccagcuuuauuggg

SEQ ID NO: 41 - RNA, 21 nt, Artificial Sequence
  siRNA
cccaauaaagcuggacaagaa

SEQ ID NO: 42 - RNA, 23 nt, Artificial Sequence
  siRNA
uucuuguccagcuuuauugggag

SEQ ID NO: 43 - RNA, 21 nt, Artificial Sequence
  siRNA
cccaauaaagcuggacaagaa

SEQ ID NO: 44 - RNA, 23 nt, Artificial Sequence
  siRNA
uucuuguccagcuuuauugggag

SEQ ID NO: 45 - RNA, 19 nt, Artificial Sequence
  siRNA
  misc_feature (19)..(19): n is Z5, and Z5 is U
uuaaaagggacaguauucn

SEQ ID NO: 46 - RNA, 19 nt, Artificial Sequence
  siRNA
  misc_feature (1)..(1): n is Z6, and Z6 is A
ngaauacugucccuuuuaa

SEQ ID NO: 47 - RNA, 19 nt, Artificial Sequence
  siRNA
  misc_feature (19)..(19): n is Z7, and Z7 is selected from A, U, G or C
uuaaaagggacaguauucn

SEQ ID NO: 48 - RNA, 19 nt, Artificial Sequence
  siRNA
  misc_feature (1)..(1): n is Z8, Z8 is a nucleotide complementary to Z7, and Z7 is selected from A, U, G or C
ngaauacugucccuuuuaa

SEQ ID NO: 49 - RNA, 19 nt, Artificial Sequence
  siRNA
  misc_feature (19)..(19): n is Z7, and Z7 is selected from A, U, G or C
uuaaaagggacaguauucn

SEQ ID NO: 50 - RNA, 21 nt, Artificial Sequence
  siRNA
  misc_feature (1)..(1): n is Z8, Z8 is a nucleotide complementary to Z7, and Z7 is selected from A, U, G or C
ngaauacugucccuuuuaagc

SEQ ID NO: 51 - RNA, 21 nt, Artificial Sequence
  siRNA
  misc_feature (21)..(21): n is Z7, and Z7 is selected from A, U, G or C
gcuuaaaagggacaguauucn

SEQ ID NO: 52 - RNA, 23 nt, Artificial Sequence
  siRNA
  misc_feature (1)..(1): n is Z8, Z8 is a nucleotide complementary to Z7, and Z7 is selected from A, U, G or C
ngaauacugucccuuuuaagcaa

SEQ ID NO: 53 - RNA, 19 nt, Artificial Sequence
  siRNA
uuaaaagggacaguauucu

SEQ ID NO: 54 - RNA, 21 nt, Artificial Sequence
  siRNA
agaauacugucccuuuuaagc

SEQ ID NO: 55 - RNA, 21 nt, Artificial Sequence
  siRNA
gcuuaaaagggacaguauucu

SEQ ID NO: 56 - RNA, 23 nt, Artificial Sequence
  siRNA
agaauacugucccuuuuaagcaa

SEQ ID NO: 57 - RNA, 19 nt, Artificial Sequence
  siRNA
uuaaaagggacaguauucu

SEQ ID NO: 58 - RNA, 21 nt, Artificial Sequence
  siRNA
agaauacugucccuuuuaagc

SEQ ID NO: 59 - RNA, 19 nt, Artificial Sequence
  siRNA
uuaaaagggacaguauucu

SEQ ID NO: 60 - RNA, 21 nt, Artificial Sequence
  siRNA
agaauacugucccuuuuaagc

SEQ ID NO: 61 - RNA, 21 nt, Artificial Sequence
  siRNA
gcuuaaaagggacaguauucu

SEQ ID NO: 62 - RNA, 23 nt, Artificial Sequence
  siRNA
agaauacugucccuuuuaagcaa

SEQ ID NO: 63 - RNA, 21 nt, Artificial Sequence
  siRNA
gcuuaaaagggacaguauucu

SEQ ID NO: 64 - RNA, 23 nt, Artificial Sequence
  siRNA
agaauacugucccuuuuaagcaa

SEQ ID NO: 65 - RNA, 19 nt, Artificial Sequence
  siRNA
uuaaaagggacaguauucu

SEQ ID NO: 66 - RNA, 21 nt, Artificial Sequence
  siRNA
agaauacugucccuuuuaagc

SEQ ID NO: 67 - RNA, 19 nt, Artificial Sequence
  siRNA
uuaaaagggacaguauucu

SEQ ID NO: 68 - RNA, 21 nt, Artificial Sequence
  siRNA
agaauacugucccuuuuaagc

SEQ ID NO: 69 - RNA, 21 nt, Artificial Sequence
  siRNA
gcuuaaaagggacaguauucu

SEQ ID NO: 70 - RNA, 23 nt, Artificial Sequence
  siRNA
agaauacugucccuuuuaagcaa

SEQ ID NO: 71 - RNA, 21 nt, Artificial Sequence
  siRNA
gcuuaaaagggacaguauucu

SEQ ID NO: 72 - RNA, 23 nt, Artificial Sequence
  siRNA
agaauacugucccuuuuaagcaa

SEQ ID NO: 73 - RNA, 19 nt, Artificial Sequence
  siRNA
uuaaaagggacaguauucu

SEQ ID NO: 74 - RNA, 21 nt, Artificial Sequence
  siRNA
agaauacugucccuuuuaagc

SEQ ID NO: 75 - RNA, 19 nt, Artificial Sequence
  siRNA
uuaaaagggacaguauucu

SEQ ID NO: 76 - RNA, 21 nt, Artificial Sequence
  siRNA
agaauacugucccuuuuaagc

SEQ ID NO: 77 - RNA, 21 nt, Artificial Sequence
  siRNA
gcuuaaaagggacaguauucu

SEQ ID NO: 78 - RNA, 23 nt, Artificial Sequence
  siRNA
agaauacugucccuuuuaagcaa

SEQ ID NO: 79 - RNA, 21 nt, Artificial Sequence
  siRNA
gcuuaaaagggacaguauucu

SEQ ID NO: 80 - RNA, 23 nt, Artificial Sequence
  siRNA
agaauacugucccuuuuaagcaa

SEQ ID NO: 81 - RNA, 19 nt, Artificial Sequence
  siRNA
uuaaaagggacaguauucu

SEQ ID NO: 82 - RNA, 21 nt, Artificial Sequence
  siRNA
agaauacugucccuuuuaagc

SEQ ID NO: 83 - RNA, 19 nt, Artificial Sequence
  siRNA
uuaaaagggacaguauucu

SEQ ID NO: 84 - RNA, 21 nt, Artificial Sequence
  siRNA
agaauacugucccuuuuaagc

SEQ ID NO: 85 - RNA, 21 nt, Artificial Sequence
  siRNA
gcuuaaaagggacaguauucu

SEQ ID NO: 86 - RNA, 23 nt, Artificial Sequence
  siRNA
agaauacugucccuuuuaagcaa

SEQ ID NO: 87 - RNA, 21 nt, Artificial Sequence
  siRNA
gcuuaaaagggacaguauucu

SEQ ID NO: 88 - RNA, 23 nt, Artificial Sequence
  siRNA
agaauacugucccuuuuaagcaa

SEQ ID NO: 89 - RNA, 21 nt, Artificial Sequence
  siRNA
agaauacugucccuuuuaauu

SEQ ID NO: 90 - RNA, 21 nt, Artificial Sequence
  siRNA
agaauacugucccuuuuaauu

SEQ ID NO: 91 - RNA, 23 nt, Artificial Sequence
  siRNA
agaauacugucccuuuuaagcuu

SEQ ID NO: 92 - RNA, 23 nt, Artificial Sequence
  siRNA
agaauacugucccuuuuaagcuu

SEQ ID NO: 93 - RNA, 21 nt, Artificial Sequence
  siRNA
agaauacugucccuuuuaauu

SEQ ID NO: 94 - RNA, 21 nt, Artificial Sequence
  siRNA
agaauacugucccuuuuaauu

SEQ ID NO: 95 - RNA, 23 nt, Artificial Sequence
  siRNA
agaauacugucccuuuuaagcuu

SEQ ID NO: 96 - RNA, 23 nt, Artificial Sequence
  siRNA
agaauacugucccuuuuaagcuu

SEQ ID NO: 97 - RNA, 21 nt, Artificial Sequence
  siRNA
agaauacugucccuuuuaauu

SEQ ID NO: 98 - RNA, 21 nt, Artificial Sequence
  siRNA
agaauacugucccuuuuaauu

SEQ ID NO: 99 - RNA, 23 nt, Artificial Sequence
  siRNA
agaauacugucccuuuuaagcuu

SEQ ID NO: 100 - RNA, 23 nt, Artificial Sequence
  siRNA
agaauacugucccuuuuaagcuu

SEQ ID NO: 101 - RNA, 21 nt, Artificial Sequence
  siRNA
agaauacugucccuuuuaauu

SEQ ID NO: 102 - RNA, 21 nt, Artificial Sequence
  siRNA
agaauacugucccuuuuaauu

SEQ ID NO: 103 - RNA, 23 nt, Artificial Sequence
  siRNA
agaauacugucccuuuuaagcuu

SEQ ID NO: 104 - RNA, 23 nt, Artificial Sequence
  siRNA
agaauacugucccuuuuaagcuu

SEQ ID NO: 105 - RNA, 19 nt, Artificial Sequence
  siRNA
  misc_feature (19)..(19): n is Z9, and Z9 is U
ggacaguauucucagugcn

SEQ ID NO: 106 - RNA, 19 nt, Artificial Sequence
  siRNA
  misc_feature (1)..(1): n is Z10, and Z10 is A
ngcacugagaauacugucc

SEQ ID NO: 107 - RNA, 19 nt, Artificial Sequence
  siRNA
  misc_feature (19)..(19): n is Z11, and Z11 is selected from A, U, G or C
ggacaguauucucagugcn

SEQ ID NO: 108 - RNA, 19 nt, Artificial Sequence
  siRNA
  misc_feature (1)..(1): n is Z12, Z12 is a nucleotide complementary to Z11, and Z11 is selected from A, U, G or C
ngcacugagaauacugucc

SEQ ID NO: 109 - RNA, 19 nt, Artificial Sequence
  siRNA
  misc_feature (19)..(19): n is Z11, and Z11 is selected from A, U, G or C
ggacaguauucucagugcn

SEQ ID NO: 110 - RNA, 21 nt, Artificial Sequence
  siRNA
  misc_feature (1)..(1): n is Z12, Z12 is a nucleotide complementary to Z11, and Z11 is selected from A, U, G or C
ngcacugagaauacugucccu

SEQ ID NO: 111 - RNA, 21 nt, Artificial Sequence
  siRNA
  misc_feature (21)..(21): n is Z11, and Z11 is selected from A, U, G or C
agggacaguauucucagugcn

SEQ ID NO: 112 - RNA, 23 nt, Artificial Sequence
  siRNA
  misc_feature (1)..(1): n is Z12, Z12 is a nucleotide complementary to Z11, and Z11 is selected from A, U, G or C
ngcacugagaauacugucccuuu

SEQ ID NO: 113 - RNA, 19 nt, Artificial Sequence
  siRNA
ggacaguauucucagugcu

SEQ ID NO: 114 - RNA, 21 nt, Artificial Sequence
  siRNA
agcacugagaauacugucccu

SEQ ID NO: 115 - RNA, 21 nt, Artificial Sequence
  siRNA
agggacaguauucucagugcu

SEQ ID NO: 116 - RNA, 23 nt, Artificial Sequence
  siRNA
agcacugagaauacugucccuuu

SEQ ID NO: 117 - RNA, 19 nt, Artificial Sequence
  siRNA
ggacaguauucucagugcu

SEQ ID NO: 118 - RNA, 21 nt, Artificial Sequence
  siRNA
agcacugagaauacugucccu

SEQ ID NO: 119 - RNA, 19 nt, Artificial Sequence
  siRNA
ggacaguauucucagugcu

SEQ ID NO: 120 - RNA, 21 nt, Artificial Sequence
  siRNA
agcacugagaauacugucccu

SEQ ID NO: 121 - RNA, 21 nt, Artificial Sequence
  siRNA
agggacaguauucucagugcu

SEQ ID NO: 122 - RNA, 23 nt, Artificial Sequence
  siRNA
agcacugagaauacugucccuuu

SEQ ID NO: 123 - RNA, 21 nt, Artificial Sequence
  siRNA
agggacaguauucucagugcu

SEQ ID NO: 124 - RNA, 23 nt, Artificial Sequence
  siRNA
agcacugagaauacugucccuuu

SEQ ID NO: 125 - RNA, 19 nt, Artificial Sequence
  siRNA
ggacaguauucucagugcu

SEQ ID NO: 126 - RNA, 21 nt, Artificial Sequence
  siRNA
agcacugagaauacugucccu

SEQ ID NO: 127 - RNA, 19 nt, Artificial Sequence
  siRNA
ggacaguauucucagugcu

SEQ ID NO: 128 - RNA, 21 nt, Artificial Sequence
  siRNA
agcacugagaauacugucccu

SEQ ID NO: 129 - RNA, 21 nt, Artificial Sequence
  siRNA
agggacaguauucucagugcu

SEQ ID NO: 130 - RNA, 23 nt, Artificial Sequence
  siRNA
agcacugagaauacugucccuuu

SEQ ID NO: 131 - RNA, 21 nt, Artificial Sequence
  siRNA
agggacaguauucucagugcu

SEQ ID NO: 132 - RNA, 23 nt, Artificial Sequence
  siRNA
agcacugagaauacugucccuuu

SEQ ID NO: 133 - RNA, 19 nt, Artificial Sequence
  siRNA
ggacaguauucucagugcu

SEQ ID NO: 134 - RNA, 21 nt, Artificial Sequence
  siRNA
agcacugagaauacugucccu

SEQ ID NO: 135 - RNA, 19 nt, Artificial Sequence
  siRNA
ggacaguauucucagugcu

SEQ ID NO: 136 - RNA, 21 nt, Artificial Sequence
  siRNA
agcacugagaauacugucccu

SEQ ID NO: 137 - RNA, 21 nt, Artificial Sequence
  siRNA
agggacaguauucucagugcu

SEQ ID NO: 138 - RNA, 23 nt, Artificial Sequence
  siRNA
agcacugagaauacugucccuuu

SEQ ID NO: 139 - RNA, 21 nt, Artificial Sequence
  siRNA
agggacaguauucucagugcu

SEQ ID NO: 140 - RNA, 23 nt, Artificial Sequence
  siRNA
agcacugagaauacugucccuuu

SEQ ID NO: 141 - RNA, 19 nt, Artificial Sequence
  siRNA
ggacaguauucucagugcu

SEQ ID NO: 142 - RNA, 21 nt, Artificial Sequence
  siRNA
agcacugagaauacugucccu

SEQ ID NO: 143 - RNA, 19 nt, Artificial Sequence
  siRNA
ggacaguauucucagugcu

SEQ ID NO: 144 - RNA, 21 nt, Artificial Sequence
  siRNA
agcacugagaauacugucccu

SEQ ID NO: 145 - RNA, 21 nt, Artificial Sequence
  siRNA
agggacaguauucucagugcu

SEQ ID NO: 146 - RNA, 23 nt, Artificial Sequence
  siRNA
agcacugagaauacugucccuuu

SEQ ID NO: 147 - RNA, 21 nt, Artificial Sequence
  siRNA
agggacaguauucucagugcu

SEQ ID NO: 148 - RNA, 23 nt, Artificial Sequence
  siRNA
agcacugagaauacugucccuuu

SEQ ID NO: 149 - RNA, 21 nt, Artificial Sequence
  siRNA
  misc_feature (1)..(1): n is Z8, Z8 is a nucleotide complementary to Z7, and Z7 is selected from A, U, G or C
ngaauacugucccuuuuaauu

SEQ ID NO: 150 - RNA, 23 nt, Artificial Sequence
  siRNA
  misc_feature (1)..(1): n is Z8, Z8 is a nucleotide complementary to Z7, and Z7 is selected from A, U, G or C
ngaauacugucccuuuuaagcuu

SEQ ID NO: 151 - RNA, 21 nt, Artificial Sequence
  siRNA
uucuuguccagcuuuauuggg

SEQ ID NO: 152 - RNA, 21 nt, Artificial Sequence
  siRNA
uucuuguccagcuuuauuggg

SEQ ID NO: 153 - RNA, 21 nt, Artificial Sequence
  siRNA
agaauacugucccuuuuaagc

SEQ ID NO: 154 - RNA, 21 nt, Artificial Sequence
  siRNA
agaauacugucccuuuuaagc

SEQ ID NO: 155 - RNA, 21 nt, Artificial Sequence
  siRNA
agaauacugucccuuuuaauu

SEQ ID NO: 156 - RNA, 21 nt, Artificial Sequence
  siRNA
agcacugagaauacugucccu

SEQ ID NO: 157 - RNA, 21 nt, Artificial Sequence
  siRNA
agcacugagaauacugucccu

SEQ ID NO: 158 - RNA, 21 nt, Artificial Sequence
  siRNA
uucuuguccagcuuuauuggg

SEQ ID NO: 159 - RNA, 21 nt, Artificial Sequence
  siRNA
agaauacugucccuuuuaagc

SEQ ID NO: 160 - RNA, 21 nt, Artificial Sequence
  siRNA
agcacugagaauacugucccu

SEQ ID NO: 161 - RNA, 19 nt, Artificial Sequence
  siRNA
uucuccgaacgugucacgu

SEQ ID NO: 162 - RNA, 21 nt, Artificial Sequence
  siRNA
acgugacacguucggagaacu

SEQ ID NO: 163 - DNA, 532 bp, Artificial Sequence
  Target sequence 1
tgctcagttcatccctagaggcagctgctccaggaacagaggtgccatgcagccccgggtactccttgttgttgccctcctggcgctcctggcctctgcccgagcttcagaggccgaggatgcctcccttctcagcttcatgcagggttacatgaagcacgccaccaagaccgccaaggatgcactgagcagcgtgcaggagtcccaggtggcccagcaggccaggggctgggtgaccgatggcttcagttccctgaaagactactggagcaccgttaaggacaagttctctgagttctgggatttggaccctgaggtcagaccaacttcagccgtggctgcctgagacctcaataccccaagtccacctgcctatccatcctgcgagctccttgggtcctgcaatctccagggctgcccctgtaggttgcttaaaagggacagtattctcagtgctctcctaccccacctcatgcctggcccccctccaggcatgctggcctcccaataaagctggacaagaagctgctat

SEQ ID NO: 164 - DNA, 38 bp, Artificial Sequence
  Target sequence 2
ttgcttaaaagggacagtattctcagtgctctcctacc

SEQ ID NO: 165 - DNA, 21 bp, Artificial Sequence
  Target sequence 3
taggcccctttcaagtattct

SEQ ID NO: 166 - DNA, 21 bp, Artificial Sequence
  Target sequence 4
agaatactgtcccttttaagc

SEQ ID NO: 167 - DNA, 21 bp, Artificial Sequence
  Target sequence 5
ctccgcagtgaaattttaagc

SEQ ID NO: 168 - DNA, 21 bp, Artificial Sequence
  Target sequence 6
ctttcactgcggatcagtgct

SEQ ID NO: 169 - DNA, 21 bp, Artificial Sequence
  Target sequence 7
agcactgagaatactgtccct

SEQ ID NO: 170 - DNA, 21 bp, Artificial Sequence
  Target sequence 8
ctacagtctccgcctgtccct